European Patent Application EP 4 592 383 A2, published July 30, 2025. Title: POLY-DONOR CD4+ T CELLS EXPRESSING IL-10 AND USES THEREOF. Applicant: TR1X, INC. Application EP. The sequence listing filed with the application follows.

SEQUENCE LISTING (5 sequences)

SEQ ID NO: 1 - protein, 178 aa, Homo sapiens
MHSSALLCCLVLLTGVRASPGQGTQSENSCTHFPGNLPNMLRDLRDAFSRVKTFFQMKDQLDNLLLKESLLEDFKGYLGCQALSEMIQFYLEEVMPQAENQDPDIKAHVNSLGENLKTLRLRLRRCHRFLPCENKSKAVEQVKNAFNKLQEKGIYKAMSEFDIFINYIEAYMTMKIRN

SEQ ID NO: 2 - DNA, 498 bp, Homo sapiens
  source 1..498: mol_type = other DNA
ggggtgagggccagcccaggccagggcacccagtctgagaacagctgcacccacttcccaggcaacctgcctaacatgcttcgagatctccgagatgccttcagcagagtgaagactttctttcaaatgaaggatcagctggacaacttgttgttaaaggagtccttgctggaggactttaagggttacctgggttgccaagccttgtctgagatgatccagttttacctggaggaggtgatgccccaagctgagaaccaagacccagacatcaaggcgcatgtgaactccctgggggagaacctgaagaccctcaggctgaggctacggcgctgtcatcgatttcttccctgtgaaaacaagagcaaggccgtggagcaggtgaagaatgcctttaataagctccaagagaaaggcatctacaaagccatgagtgagtttgacatcttcatcaactacatagaagcctacatgacaatgaagatacgaaactgagtc

SEQ ID NO: 3 - protein, 281 aa, synthetic construct
LEDPPVPPLEGYVGHKAHNHSSQDGAIDRDEVVGGASGHHGLGAAHHCGHHTCHRAGYEVLFWRCLRLLGAGGCAVRALWGCGPCNPTARDLLALGVGPACALAELALGVLAHGAGQARVHVVGLVGIRAVGALLAHGVLLVLAGEHEARARLAHAARLAAPSRLILVVAVGAAAHGVVGLHARRRHALEPHALGARLARLGRAHHVGERHAVQAGLTHGLVGSTRLGHTLAQVAGFAALTAVCVQACGACLLGTSKGHPQKQQQQQARPVHGAAGGTCPH

SEQ ID NO: 4 - DNA, 843 bp, synthetic construct
  source 1..843: mol_type = other DNA
ctagaggatccccctgttccacctcttgaaggctatgtaggccacaaggcccacaaccacagcagccaggatggagcaatagacagggatgaggttgtcggtggtgcctcgggtcaccacgggctgggagctgcccatcactgtggtcaccacacctgccaccgtgctggctatgaggtcttgttctggaggtgcctcaggctcctgggtgctgggggctgtgctgtccgagccctctgggggtgtggaccgtgtaatccaacggccagggatctcctcgcactcggcgtcggcccagcgtgtgcactcgcggagctggcgctcggtgtcctcgcacacggtgcagggcaggcacgggtccacgtggttggcctcgtcggaatacgtgccgtcggggcactcctcgcacacggtgttctgcttgtcctggcaggagaacacgaggcccgagcccgcctcgcacacgcggcacgcctcgcagcgcccagtcgtctcatcctggtagtagccgtaggcgcagcggcacacggcgtcgtcggcctccacgcacggcgccgacatgctctggagccccacgcactcggtgcacggcttgcacggctcggtcgcgctcaccacgtcggagaacgtcacgctgtccaggcagggctcacacacggtctggttggctccacaaggctgggccacaccctcgcccaggttgcaggctttgcagcactcaccgctgtgtgtgtacaggcctgtggggcatgcctccttggcacctccaagggacacccccagaagcagcaacagcagcaggcgcggcccgtccatggcgcggccggtggcacctgcccccat

SEQ ID NO: 5 - DNA, 9025 bp, synthetic construct
  source 1..9025: mol_type = other DNA
aaatttcacaaataaagcatttttttcactgcattctagttgtggtttgtccaaactcatcaatgtatcttatcatgtctggctctagctatcccgcccctaactccgcccagttccgcccattctccgccccatggctgactaattttttttatttatgcagaggccgaggccgcctcggcctctgagctattccagaagtagtgaggaggcttttttggaggcctaggcttttgcgtcgagacgtacccaattcgccctatagtgagtcgtattacgcgcgctcactggccgtcgttttacaacgtcgtgactgggaaaaccctggcgttacccaacttaatcgccttgcagcacatccccctttcgccagctggcgtaatagcgaagaggcccgcaccgatcgcccttcccaacagttgcgcagcctgaatggcgaatggcgcgacgcgccctgtagcggcgcattaagcgcggcgggtgtggtggttacgcgcagcgtgaccgctacacttgccagcgccctagcgcccgctcctttcgctttcttcccttcctttctcgccacgttcgccggctttccccgtcaagctctaaatcgggggctccctttagggttccgatttagtgctttacggcacctcgaccccaaaaaacttgattagggtgatggttcacgtagtgggccatcgccctgatagacggtttttcgccctttgacgttggagtccacgttctttaatagtggactcttgttccaaactggaacaacactcaaccctatctcggtctattcttttgatttataagggattttgccgatttcggcctattggttaaaaaatgagctgatttaacaaaaatttaacgcgaattttaacaaaatattaacgtttacaatttcccaggtggcacttttcggggaaatgtgcgcggaacccctatttgtttatttttctaaatacattcaaatatgtatccgctcatgagacaataaccctgataaatgcttcaataatattgaaaaaggaagagtatgagtattcaacatttccgtgtcgcccttattcccttttttgcggcattttgccttcctgtttttgctcacccagaaacgctggtgaaagtaaaagatgctgaagatcagttgggtgcacgagtgggttacatcgaactggatctcaacagcggtaagatccttgagagttttcgccccgaagaacgttttccaatgatgagcacttttaaagttctgctatgtggcgcggtattatcccgtattgacgccgggcaagagcaactcggtcgccgcatacactattctcagaatgacttggttgagtactcaccagtcacagaaaagcatcttacggatggcatgacagtaagagaattatgcagtgctgccataaccatgagtgataacactgcggccaacttacttctgacaacgatcggaggaccgaaggagctaaccgcttttttgcacaacatgggggatcatgtaactcgccttgatcgttgggaaccggagctgaatgaagccataccaaacgacgagcgtgacaccacgatgcctgtagcaatggcaacaacgttgcgcaaactattaactggcgaactacttactctagcttcccggcaacaattaatagactggatggaggcggataaagttgcaggaccacttctgcgctcggcccttccggctggctggtttattgctgataaatctggagccggtgagcgtgggtctcgcggtatcattgcagcactggggccagatggtaagccctcccgtatcgtagttatctacacgacggggagtcaggcaactatggatgaacgaaatagacagatcgctgagataggtgcctcactgattaagcattggtaactgtcagaccaagtttactcatatatactttagattgatttaaaacttcatttttaatttaaaaggatctaggtgaagatcctttttgataatctcatgaccaaaatcccttaacgtgagttttcgttccactgagcgtcagaccccgtagaaaagatcaaaggatcttcttgagatcctttttttctgcgcgtaatctgctgcttgcaaacaaaaaaaccaccgctaccagcggtggtttgtttgccggatcaagagctaccaactctttttccgaaggtaactggcttcagcagagcgcagataccaaatactgtccttctagtgtagccgtagttaggccaccacttcaagaactctgtagcaccgcctacatacctcgctctgctaatcctgttaccagtggctgctgccagtggcgataagtcgtgtcttaccgggttggactcaagacgatagttaccggataaggcgcagcggtcgggctgaacggggggttcgtgcacacagcccagcttggagcgaacgacctacaccgaactgagatacctacagcgtgagctatgagaaagcgccacgcttcccgaagggagaaaggcggacaggtatccggtaagcggcagggtcggaacaggagagcgcacgagggagcttccagggggaaacgcctggtatctttatagtcctgtcgggtttcgccacctctgacttgagcgtcgatttttgtgatgctcgtcaggggggcggagcctatggaaaaacgccagcaacgcggcctttttacggttcctggccttttgctggccttttgctcacatgttctttcctgcgttatcccctgattctgtggataaccgtattaccgcctttgagtgagctgataccgctcgccgcagccgaacgaccgagcgcagcgagtcagtgagcgaggaagcggaagagcgcccaatacgcaaaccgcctctccccgcgcgttggccgattcattaatgcagctggcacgacaggtttcccgactggaaagcgggcagtgagcgcaacgcaattaatgtgagttagctcactcattaggcaccccaggctttacactttatgcttccggctcgtatgttgtgtggaattgtgagcggataacaatttcacacaggaaacagctatgaccatgattacgccaagcgcgcaattaaccctcactaaagggaacaaaagctggagctgcaagcttggccattgcatacgttgtatccatatcataatatgtacatttatattggctcatgtccaacattaccgccatgttgacattgattattgactagttattaatagtaatcaattacggggtcattagttcatagcccatatatggagttccgcgttacataacttacggtaaatggcccgcctggctgaccgcccaacgacccccgcccattgacgtcaataatgacgtatgttcccatagtaacgccaatagggactttccattgacgtcaatgggtggagtatttacggtaaactgcccacttggcagtacatcaagtgtatcatatgccaagtacgccccctattgacgtcaatgacggtaaatggcccgcctggcattatgcccagtacatgaccttatgggactttcctacttggcagtacatctacgtattagtcatcgctattaccatggtgatgcggttttggcagtacatcaatgggcgtggatagcggtttgactcacggggatttccaagtctccaccccattgacgtcaatgggagtttgttttggcaccaaaatcaacgggactttccaaaatgtcgtaacaactccgccccattgacgcaaatgggcggtaggcgtgtacggtgggaggtctatataagcagagctcgtttagtgaaccggggtctctctggttagaccagatctgagcctgggagctctctggctaactagggaacccactgcttaagcctcaataaagcttgccttgagtgcttcaagtagtgtgtgcccgtctgttgtgtgactctggtaactagagatccctcagacccttttagtcagtgtggaaaatctctagcagtggcgcccgaacagggacctgaaagcgaaagggaaaccagagctctctcgacgcaggactcggcttgctgaagcgcgcacggcaagaggcgaggggcggcgactggtgagtacgccaaaaattttgactagcggaggctagaaggagagagatgggtgcgagagcgtcagtattaagcgggggagaattagatcgcgatgggaaaaaattcggttaaggccagggggaaagaaaaaatataaattaaaacatatagtatgggcaagcagggagctagaacgattcgcagttaatcctggcctgttagaaacatcagaaggctgtagacaaatactgggacagctacaaccatcccttcagacaggatcagaagaacttagatcattatataatacagtagcaaccctctattgtgtgcatcaaaggatagagataaaagacaccaaggaagctttagacaagatagaggaagagcaaaacaaaagtaagaccaccgcacagcaagcggccgctgatcttcagacctggaggaggagatatgagggacaattggagaagtgaattatataaatataaagtagtaaaaattgaaccattaggagtagcacccaccaaggcaaagagaagagtggtgcagagagaaaaaagagcagtgggaataggagctttgttccttgggttcttgggagcagcaggaagcactatgggcgcagcctcaatgacgctgacggtacaggccagacaattattgtctggtatagtgcagcagcagaacaatttgctgagggctattgaggcgcaacagcatctgttgcaactcacagtctggggcatcaagcagctccaggcaagaatcctggctgtggaaagatacctaaaggatcaacagctcctggggatttggggttgctctggaaaactcatttgcaccactgctgtgccttggaatgctagttggagtaataaatctctggaacagattggaatcacacgacctggatggagtgggacagagaaattaacaattacacaagcttaatacactccttaattgaagaatcgcaaaaccagcaagaaaagaatgaacaagaattattggaattagataaatgggcaagtttgtggaattggtttaacataacaaattggctgtggtatataaaattattcataatgatagtaggaggcttggtaggtttaagaatagtttttgctgtactttctatagtgaatagagttaggcagggatattcaccattatcgtttcagacccacctcccaaccccgaggggacccgacaggcccgaaggaatagaagaagaaggtggagagagagacagagacagatccattcgattagtgaacggatctcgacggtatcggttaacttttaaaagaaaaggggggattggggggtacagtgcaggggaaagaatagtagacataatagcaacagacatacaaactaaagaattacaaaaacaaattacaaaaattcaaaattttatcgatcacgagactagcctcgagagatctgatcataatcagccataccacatttgtagaggttttacttgctttaaaaaacctcccacacctccccctgaacctgaaacataaaatgaatgcaattgttgttgttaacttgtttattgcagcttataatggttacaaataaggcaatagcatcacaaatttcacaaataaggcatttttttcactgcattctagttttggtttgtccaaactcatcaatgtatcttatcatgtctggatctcaaatccctcggaagctgcgcctgtcatcgaattcctgcagcccggtgcatgactaagctagctcagttagcctcccccatctcccctagaggatccccctgttccacctcttgaaggctatgtaggccacaaggcccacaaccacagcagccaggatggagcaatagacagggatgaggttgtcggtggtgcctcgggtcaccacgggctgggagctgcccatcactgtggtcaccacacctgccaccgtgctggctatgaggtcttgttctggaggtgcctcaggctcctgggtgctgggggctgtgctgtccgagccctctgggggtgtggaccgtgtaatccaacggccagggatctcctcgcactcggcgtcggcccagcgtgtgcactcgcggagctggcgctcggtgtcctcgcacacggtgcagggcaggcacgggtccacgtggttggcctcgtcggaatacgtgccgtcggggcactcctcgcacacggtgttctgcttgtcctggcaggagaacacgaggcccgagcccgcctcgcacacgcggcacgcctcgcagcgcccagtcgtctcatcctggtagtagccgtaggcgcagcggcacacggcgtcgtcggcctccacgcacggcgccgacatgctctggagccccacgcactcggtgcacggcttgcacggctcggtcgcgctcaccacgtcggagaacgtcacgctgtccaggcagggctcacacacggtctggttggctccacaaggctgggccacaccctcgcccaggttgcaggctttgcagcactcaccgctgtgtgtgtacaggcctgtggggcatgcctccttggcacctccaagggacacccccagaagcagcaacagcagcaggcgcggcccgtccatggcgcggccggtggcacctgcccccatcgcccgcctcccgcggcagcgctcgacttccagctcggtccgctttgcggactgatggggctgcgctgcgctgcgctccagcgccccccctgcccgccggagctggccgcggcccgaattccgcggaggctggatcggtcccggtgtcttctatggaggtcaaaacagcgtggatggcgtctccaggcgatctgacggttcactaaacgagctctgcttatataggcctcccaccgtacacgcctaccctcgagaagcttgatatcgaattcccacggggttggggttgcgccttttccaaggcagccctgggtttgcgcagggacgcggctgctctgggcgtggttccgggaaacgcagcggcgccgaccctgggtctcgcacattcttcacgtccgttcgcagcgtcacccggatcttcgccgctacccttgtgggccccccggcgacgcttcctgctccgcccctaagtcgggaaggttccttgcggttcgcggcgtgccggacgtgacaaacggaagccgcacgtctcactagtaccctcgcagacggacagcgccagggagcaatggcagcgcgccgaccgcgatgggctgtggccaatagcggctgctcagcggggcgcgccgagagcagcggccgggaaggggcggtgcgggaggcggggtgtggggcggtagtgtgggccctgttcctgcccgcgcggtgttccgcattctgcaagcctccggagcgcacgtcggcagtcggctccctcgttgaccgaatcaccgacctctctccccagggggatccccggtctgcaggaattcatgcacagctcagcactgctctgttgcctggtcctcctgactggggtgagggccagcccaggccagggcacccagtctgagaacagctgcacccacttcccaggcaacctgcctaacatgcttcgagatctccgagatgccttcagcagagtgaagactttctttcaaatgaaggatcagctggacaacttgttgttaaaggagtccttgctggaggactttaagggttacctgggttgccaagccttgtctgagatgatccagttttacctggaggaggtgatgccccaagctgagaaccaagacccagacatcaaggcgcatgtgaactccctgggggagaacctgaagaccctcaggctgaggctacggcgctgtcatcgatttcttccctgtgaaaacaagagcaaggccgtggagcaggtgaagaatgcctttaataagctccaagagaaaggcatctacaaagccatgagtgagtttgacatcttcatcaactacatagaagcctacatgacaatgaagatacgaaactgagtcgagaatcaacctctggattacaaaatttgtgaaagattgactggtattcttaactatgttgctccttttacgctatgtggatacgctgctttaatgcctttgtatcatgctattgcttcccgtatggctttcattttctcctccttgtataaatcctggttgctgtctctttatgaggagttgtggcccgttgtcaggcaacgtggcgtggtgtgcactgtgtttgctgacgcaacccccactggttggggcattgccaccacctgtcagctcctttccgggactttcgctttccccctccctattgccacggcggaactcatcgccgcctgccttgcccgctgctggacaggggctcggctgttgggcactgacaattccgtggtgttgtcggggaagctgacgtcctttccatggctgctcgcctgtgttgccacctggattctgcgcgggacgtccttctgctacgtcccttcggccctcaatccagcggaccttccttcccgcggcctgctgccggctctagagcctcttccgcgtcttcgccttcccgggtcgagctcggtacctttaagaccaatgacttacaaggcagctgtagatcttagccactttttaaaagaaaaggggggactggaagggctaattcactcccaacgaagacaagatctgctttttgcttgtactgggtctctctggttagaccagatctgagcctgggagctctctggctaactagggaacccactgcttaagcctcaataaagcttgccttgagtgcttcaagtagtgtgtgcccgtctgttgtgtgactctggtaactagagatccctcagacccttttagtcagtgtggaaaatctctagcagtagtagttcatgtcatcttattattcagtatttataacttgcaaagaaatgaatatcagagagtgagaggaacttgtttattgcagcttataatggttacaaataaagcaatagcatcac